European Patent Application EP 4 674 430 A1, published January 7, 2026. Title: EDITED CYTOTOXIC CELLS WITH CHIMERIC ANTIGEN RECEPTORS TARGETING CD30 FOR THE TREATMENT OF VIRAL INFECTIONS AND ASSOCIATED PATHOLOGIES. Applicant: Universität zu Köln. The sequence listing filed with the application follows.

SEQUENCE LISTING (53 sequences)

SEQ ID NO: 1 - protein, 5 aa, synthetic construct
TYTIH

SEQ ID NO: 2 - protein, 17 aa, synthetic construct
YINPSSGCSDYNQNFKG

SEQ ID NO: 3 - protein, 14 aa, synthetic construct
RADYGNYEYTWFAY

SEQ ID NO: 4 - protein, 11 aa, synthetic construct
KASQNVGTNVA

SEQ ID NO: 5 - protein, 7 aa, synthetic construct
SASYRYS

SEQ ID NO: 6 - protein, 9 aa, synthetic construct
QQYHTYPLT

SEQ ID NO: 7 - protein, 127 aa, synthetic construct
RMAQVQLQQSGAELARPGASVKMSCKASGYTFTTYTIHWVRRRPGHDLEWIGYINPSSGCSDYNQNFKGKTTLTADKSSNTAYMQLNSLTSEDSAVYYCARRADYGNYEYTWFAYWGQGTTVTVSSS

SEQ ID NO: 8 - protein, 111 aa, synthetic construct
VIELTQSPKFMSTSVGDRVNVTYKASQNVGTNVAWFQQKPGQSPKVLIYSASYRYSGVPDRFTGSGSGTDFTLTISNVQSEDLAEYFCQQYHTYPLTFGGGTKLEIKRSDP

SEQ ID NO: 9 - protein, 5 aa, synthetic construct
AYYWS

SEQ ID NO: 10 - protein, 16 aa, synthetic construct
DINHGGGTNYNPSLKS

SEQ ID NO: 11 - protein, 4 aa, synthetic construct
LTAY

SEQ ID NO: 12 - protein, 11 aa, synthetic construct
RASQGISSWLT

SEQ ID NO: 13 - protein, 7 aa, synthetic construct
AASSLQS

SEQ ID NO: 14 - protein, 9 aa, synthetic construct
QQYDSYPIT

SEQ ID NO: 15 - protein, 112 aa, synthetic construct
QVQLQQWGAGLLKPSETLSLTCAVYGGSFSAYYWSWIRQPPGKGLEWIGDINHGGGTNYNPSLKSRVTISVDTSKNQFSLKLNSVTAADTAVYYCASLTAYWGQGSLVTVSS

SEQ ID NO: 16 - protein, 107 aa, synthetic construct
DIQMTQSPTSLSASVGDRVTITCRASQGISSWLTWYQQKPEKAPKSLIYAASSLQSGVPSRFSGSGSGTDFTLTISSLQPEDFATYYCQQYDSYPITFGQGTRLEIK

SEQ ID NO: 17 - protein, 5 aa, synthetic construct
GYYWS

SEQ ID NO: 18 - protein, 16 aa, synthetic construct
EINHSGSTKYTPSLKS

SEQ ID NO: 19 - protein, 8 aa, synthetic construct
ETVYYFDL

SEQ ID NO: 20 - protein, 11 aa, synthetic construct
RASQSVSSNLA

SEQ ID NO: 21 - protein, 7 aa, synthetic construct
DASNRAT

SEQ ID NO: 22 - protein, 9 aa, synthetic construct
QQRSNWPWT

SEQ ID NO: 23 - skipped

SEQ ID NO: 24 - protein, 107 aa, synthetic construct
EIVLTQSPATLSLSPGERATLSCRASQSVSSNLAWYQQKPGQAPRLLIYDASNRATGIPARLSGSGSGTDFTLTISSLEPEDFAVYYCQQRSNWPWTFGQGTKVEIK

SEQ ID NO: 25 - DNA, 398 bp, synthetic construct
  source 1..398: mol_type = other DNA
tattaaataaaagaataagcagtattattaagtagccctgcatttcaggtttccttgagtggcaggccaggcctggccgtgaacgttcactgaaatcatggcctcttggccaagattgatagcttgtgcctgtccctgagtcccagtccatcacgagcagctggtttctaagatgctatttcccgtataaagcatgagaccgtgacttgccagccccacagagccccgcccttgtccatcactggcatctggactccagcctgggttggggcaaagagggaaatgagatcatgtcctaaccctgatcctcttgtcccacagatatccagaaccctgaccctgccgtgtaccagctgagagactctaaatccagtgacaagtctgtctgcctattcacc

SEQ ID NO: 26 - DNA, 399 bp, synthetic construct
  source 1..399: mol_type = other DNA
attttgattctcaaacaaatgtgtcacaaagtaaggattctgatgtgtatatcacagacaaaactgtgctagacatgaggtctatggacttcaagagcaacagtgctgtggcctggagcaacaaatctgactttgcatgtgcaaacgccttcaacaacagcattattccagaagacaccttcttccccagcccaggtaagggcagctttggtgccttcgcaggctgtttccttgcttcaggaatggccaggttctgcccagagctctggtcaatgatgtctaaaactcctctgattggtggtctcggccttatccattgccaccaaaaccctctttttactaagaaacagtgagccttgttctggcagtccagagaatgacacgggaaaaaagcagatg

SEQ ID NO: 27 - protein, 18 aa, synthetic construct
GSTSGSGKPGSGEGSTKG

SEQ ID NO: 28 - protein, 16 aa, synthetic construct
SGGGGSGGGGSGGGGS

SEQ ID NO: 29 - protein, 4 aa, synthetic construct
GDPA

SEQ ID NO: 30 - protein, 4 aa, synthetic construct
KDPK

SEQ ID NO: 31 - protein, 237 aa, synthetic construct
PAEPKSPDKTHTCPPCPAPPVAGPSVFLFPPKPKDTLMIARTPEVTCVVVDVSHEDPEVKFNWYVDGVEVHNAKTKPREEQYNSTYRVVSVLTVLHQDWLNGKEYKCKVSNKALPAPIEKTISKAKGQPREPQVYTLPPSRDELTKNQVSLTCLVKGFYPSDIAVEWESNGQPENNYKTTPPVLDSDGSFFLYSKLTVDKSRWQQGNVFSCSVMHEALHNHYTQKSLSLSPGKKDPK

SEQ ID NO: 32 - protein, 235 aa, synthetic construct
PAEPKSPDKTHTCPPCPAPPVAGPSVFLFPPKPKDTLMIARTPEVTCVVVDVSHEDPEVKFNWYVDGVEVHNAKTKPREEQYNSTYRVVSVLTVLHQDWLNGKEYKCKVSNKALPAPIEKTISKAKGQPREPQVYTLPPSRDELTKNQVSLTCLVKGFYPSDIAVEWESNGQPENNYKTTPPVLDSDGSFFLYSKLTVDKSRWQQGNVFSCSVMHEALHNHYTQKSLSSLSPGKK

SEQ ID NO: 33 - protein, 107 aa, synthetic construct
GQPREPQVYTLPPSRDELTKNQVSLTCLVKGFYPSDIAVEWESNGQPENNYKTTPPVLDSDGSFFLYSKLTVDKSRWQQGNVFSCSVMHEALHNHYTQKSLSLSPGK

SEQ ID NO: 34 - protein, 229 aa, synthetic construct
ESKYGPPCPPCPAPEFEGGPSVFLFPPKPKDTLMISRTPEVTCVVVDVSQEDPEVQFNWYVDGVEVHNAKTKPREEQFNSTYRVVSVLTVLHQDWLNGKEYKCKVSNKGLPSSIEKTISKAKGQPREPQVYTLPPSQEEMTKNQVSLTCLVKGFYPSDIAVEWESNGQPENNYKTTPPVLDSDGSFFLYSRLTVDKSRWQEGNVFSCSVMHEALHNHYTQKSLSLSLGK

SEQ ID NO: 35 - protein, 119 aa, synthetic construct
ESKYGPPCPPCPGQPREPQVYTLPPSQEEMTKNQVSLTCLVKGFYPSDIAVEWESNGQPENNYKTTPPVLDSDGSFFLYSRLTVDKSRWQEGNVFSCSVMHEALHNHYTQKSLSLSLGK

SEQ ID NO: 36 - protein, 12 aa, synthetic construct
ESKYGPPCPPCP

SEQ ID NO: 37 - protein, 99 aa, synthetic construct
ELPTQGTFSNVSTNVSYQETTTPSTLGSTSLHPVSQHGNEATTNITETTVKFTSTSVITSVYGNTNSSVQSQTSVISTVFTTPANVSTPETTLKPSLSP

SEQ ID NO: 38 - protein, 29 aa, synthetic construct
FWVLVVVGGVLACYSLLVTVAFIIFWVRS

SEQ ID NO: 39 - protein, 24 aa, synthetic construct
IYIWAPLAGTCGVLLLSLVITLYC

SEQ ID NO: 40 - protein, 39 aa, synthetic construct
KRSRLLHSDYMNMTPRRPGPTRKHYQPYAPPRDFAAYRS

SEQ ID NO: 41 - protein, 42 aa, synthetic construct
KRGRKKLLYIFKQPFMRPVQTTQEEDGCSCRFPEEEEGGCEL

SEQ ID NO: 42 - protein, 112 aa, synthetic construct
RVKFSRSADAPAYQQGQNQLYNELNLGRREEYDVLDKRRGRDPEMGGKPRRKNPQEGLYNELQKDKMAEAYSEIGMKGERRRGKGHDGLYQGLSTATKDTYDALHMQALPPR

SEQ ID NO: 43 - protein, 22 aa, synthetic construct
GSGATNFSLLKQAGDVEENPGP

SEQ ID NO: 44 - DNA, 232 bp, synthetic construct
  source 1..232: mol_type = other DNA
ctagagctcgctgatcagcctcgactgtgccttctagttgccagccatctgttgtttgcccctcccccgtgccttccttgaccctggaaggtgccactcccactgtcctttcctaataaaatgaggaaattgcatcgcattgtctgagtaggtgtcattctattctggggggtggggtggggcaggacagcaagggggaggattgggaagagaatagcaggcatgctgggga

SEQ ID NO: 45 - protein, 561 aa, synthetic construct
MEFGLSWLFLVAILKGVQCDIQMTQSPTSLSASVGDRVTITCRASQGISSWLTWYQQKPEKAPKSLIYAASSLQSGVPSRFSGSGSGTDFTLTISSLQPEDFATYYCQQYDSYPITFGQGTRLEIKSGGGGSGGGGSGGGGSQVQLQQWGAGLLKPSETLSLTCAVYGGSFSAYYWSWIRQPPGKGLEWIGDINHGGGTNYNPSLKSRVTISVDTSKNQFSLKLNSVTAADTAVYYCASLTAYWGQGSLVTVSSGDPAESKYGPPCPPCPGQPREPQVYTLPPSRDELTKNQVSLTCLVKGFYPSDIAVEWESNGQPENNYKTTPPVLDSDGSFFLYSKLTVDKSRWQQGNVFSCSVMHEALHNHYTQKSLSLSPGKKDPKFWVLVVVGGVLACYSLLVTVAFIIFWVRSKRSRLLHSDYMNMTPRRPGPTRKHYQPYAPPRDFAAYRSRVKFSRSADAPAYQQGQNQLYNELNLGRREEYDVLDKRRGRDPEMGGKPRRKNPQEGLYNELQKDKMAEAYSEIGMKGERRRGKGHDGLYQGLSTATKDTYDALHMQALPPR

SEQ ID NO: 46 - DNA, 2781 bp, synthetic construct
  source 1..2781: mol_type = other DNA
tattaaataaaagaataagcagtattattaagtagccctgcatttcaggtttccttgagtggcaggccaggcctggccgtgaacgttcactgaaatcatggcctcttggccaagattgatagcttgtgcctgtccctgagtcccagtccatcacgagcagctggtttctaagatgctatttcccgtataaagcatgagaccgtgacttgccagccccacagagccccgcccttgtccatcactggcatctggactccagcctgggttggggcaaagagggaaatgagatcatgtcctaaccctgatcctcttgtcccacagatatccagaaccctgaccctgccgtgtaccagctgagagactctaaatccagtgacaagtctgtctgcctattcaccggcagcggcgccaccaacttcagcctgctgaagcaggccggcgacgtggaagagaaccccgggcccatggagtttggcctgagctggctgtttctggtggccattctgaagggcgtgcagtgcgacatccagatgacccagtctccaacctcactgtctgcatctgtaggagacagagtcaccatcacttgtcgggcgagtcagggtattagcagctggttaacctggtatcagcagaaaccagagaaagcccctaagtccctgatctatgctgcatccagtttgcaaagtggggtcccatcaaggttcagcggcagtggatctgggacagatttcactctcaccatcagcagcctgcagcctgaagattttgcaacttattactgccaacagtatgatagttaccctatcaccttcggccaagggacacgactggagattaaaagcggaggcggaggaagtggtggcggaggttctggcggcggaggatctcaggtgcagctacagcagtggggcgcaggactgttgaagccttcggagaccctgtccctcacctgcgctgtctatggtgggtccttcagtgcttactactggagctggatccgccagcccccagggaaggggctggagtggattggggacatcaatcatggtggaggcaccaactacaacccgtccctcaagagtcgagtcaccatatcagtagacacgtccaagaaccagttctccctgaagctgaactctgtaaccgccgcggacacggctgtgtattactgtgcgagcctaactgcctactggggccagggaagcctggtcaccgtctcctcaggggatcccgccgagtctaaatatggcccaccttgcccaccgtgcccagggcagccccgagaaccacaggtgtacaccctgcccccatcccgggatgagctgaccaagaaccaggtcagcctgacctgcctggtcaaaggcttctatcccagcgacatcgccgtggagtgggagagcaatgggcaaccggagaacaactacaagaccacgcctcccgtgctggactccgacggctccttcttcctctacagcaagctcaccgtggacaagagcaggtggcagcaggggaacgtcttctcatgctccgtgatgcatgaggctctgcacaaccactacacgcagaagagcctctccctgtctccgggtaaaaaagatcccaaattttgggtgctggtggtggttggtggagtcctggcttgctatagcttgctagtaacagtggcctttattattttctgggtgaggagtaagaggagcaggctcctgcacagtgactacatgaacatgactccccgccgccccgggcccacccgcaagcattaccagccctatgccccaccacgcgacttcgcagcctatcgctccagagtgaagttcagcaggagcgcagacgcccccgcgtaccagcagggccagaaccagctctataacgagctcaatctaggacgaagagaggagtacgatgttttggacaagagacgtggccgggaccctgagatggggggaaagccgagaaggaagaaccctcaggaaggcctgtacaatgaactgcagaaagataagatggcggaggcctacagtgagattgggatgaaaggcgagcgccggaggggcaaggggcacgatggcctttaccagggtctcagtacagccaccaaggacacctacgacgcccttcacatgcaggccctgccccctcgctgactagagctcgctgatcagcctcgactgtgccttctagttgccagccatctgttgtttgcccctcccccgtgccttccttgaccctggaaggtgccactcccactgtcctttcctaataaaatgaggaaattgcatcgcattgtctgagtaggtgtcattctattctggggggtggggtggggcaggacagcaagggggaggattgggaagagaatagcaggcatgctggggaattttgattctcaaacaaatgtgtcacaaagtaaggattctgatgtgtatatcacagacaaaactgtgctagacatgaggtctatggacttcaagagcaacagtgctgtggcctggagcaacaaatctgactttgcatgtgcaaacgccttcaacaacagcattattccagaagacaccttcttccccagcccaggtaagggcagctttggtgccttcgcaggctgtttccttgcttcaggaatggccaggttctgcccagagctctggtcaatgatgtctaaaactcctctgattggtggtctcggccttatccattgccaccaaaaccctctttttactaagaaacagtgagccttgttctggcagtccagagaatgacacgggaaaaaagcagatg

SEQ ID NO: 47 - protein, 553 aa, synthetic construct
MEFGLSWLFLVAILKGVQCDIQMTQSPTSLSASVGDRVTITCRASQGISSWLTWYQQKPEKAPKSLIYAASSLQSGVPSRFSGSGSGTDFTLTISSLQPEDFATYYCQQYDSYPITFGQGTRLEIKSGGGGSGGGGSGGGGSQVQLQQWGAGLLKPSETLSLTCAVYGGSFSAYYWSWIRQPPGKGLEWIGDINHGGGTNYNPSLKSRVTISVDTSKNQFSLKLNSVTAADTAVYYCASLTAYWGQGSLVTVSSGDPAESKYGPPCPPCPELPTQGTFSNVSTNVSYQETTTPSTLGSTSLHPVSQHGNEATTNITETTVKFTSTSVITSVYGNTNSSVQSQTSVISTVFTTPANVSTPETTLKPSLSPKDPKFWVLVVVGGVLACYSLLVTVAFIIFWVRSKRSRLLHSDYMNMTPRRPGPTRKHYQPYAPPRDFAAYRSRVKFSRSADAPAYQQGQNQLYNELNLGRREEYDVLDKRRGRDPEMGGKPRRKNPQEGLYNELQKDKMAEAYSEIGMKGERRRGKGHDGLYQGLSTATKDTYDALHMQALPPR

SEQ ID NO: 48 - DNA, 2757 bp, synthetic construct
  source 1..2757: mol_type = other DNA
tattaaataaaagaataagcagtattattaagtagccctgcatttcaggtttccttgagtggcaggccaggcctggccgtgaacgttcactgaaatcatggcctcttggccaagattgatagcttgtgcctgtccctgagtcccagtccatcacgagcagctggtttctaagatgctatttcccgtataaagcatgagaccgtgacttgccagccccacagagccccgcccttgtccatcactggcatctggactccagcctgggttggggcaaagagggaaatgagatcatgtcctaaccctgatcctcttgtcccacagatatccagaaccctgaccctgccgtgtaccagctgagagactctaaatccagtgacaagtctgtctgcctattcaccggcagcggcgccaccaacttcagcctgctgaagcaggccggcgacgtggaagagaaccccgggcccatggagtttggcctgagctggctgtttctggtggccattctgaagggcgtgcagtgcgacatccagatgacccagtctccaacctcactgtctgcatctgtaggagacagagtcaccatcacttgtcgggcgagtcagggtattagcagctggttaacctggtatcagcagaaaccagagaaagcccctaagtccctgatctatgctgcatccagtttgcaaagtggggtcccatcaaggttcagcggcagtggatctgggacagatttcactctcaccatcagcagcctgcagcctgaagattttgcaacttattactgccaacagtatgatagttaccctatcaccttcggccaagggacacgactggagattaaaagcggaggcggaggaagtggtggcggaggttctggcggcggaggatctcaggtgcagctacagcagtggggcgcaggactgttgaagccttcggagaccctgtccctcacctgcgctgtctatggtgggtccttcagtgcttactactggagctggatccgccagcccccagggaaggggctggagtggattggggacatcaatcatggtggaggcaccaactacaacccgtccctcaagagtcgagtcaccatatcagtagacacgtccaagaaccagttctccctgaagctgaactctgtaaccgccgcggacacggctgtgtattactgtgcgagcctaactgcctactggggccagggaagcctggtcaccgtctcctcaggggatcccgccgagtctaaatatggcccaccttgcccaccgtgcccagagttacctacccagggaacattttcaaatgtttctacaaatgtatcctaccaagaaactacaacacctagtacccttggaagtaccagcctgcaccctgtgtctcaacatggcaatgaggccacaacaaacatcacagaaacgacagtcaaattcacatctacctctgtgataacctcagtttatggaaacacaaactcttctgtccagtcacagacctctgtaatcagcacagtgttcaccaccccagccaacgtttcaactccagagacaaccttgaagcctagcctgtcacctaaagatcccaaattttgggtgctggtggtggttggtggagtcctggcttgctatagcttgctagtaacagtggcctttattattttctgggtgaggagtaagaggagcaggctcctgcacagtgactacatgaacatgactccccgccgccccgggcccacccgcaagcattaccagccctatgccccaccacgcgacttcgcagcctatcgctccagagtgaagttcagcaggagcgcagacgcccccgcgtaccagcagggccagaaccagctctataacgagctcaatctaggacgaagagaggagtacgatgttttggacaagagacgtggccgggaccctgagatggggggaaagccgagaaggaagaaccctcaggaaggcctgtacaatgaactgcagaaagataagatggcggaggcctacagtgagattgggatgaaaggcgagcgccggaggggcaaggggcacgatggcctttaccagggtctcagtacagccaccaaggacacctacgacgcccttcacatgcaggccctgccccctcgctgactagagctcgctgatcagcctcgactgtgccttctagttgccagccatctgttgtttgcccctcccccgtgccttccttgaccctggaaggtgccactcccactgtcctttcctaataaaatgaggaaattgcatcgcattgtctgagtaggtgtcattctattctggggggtggggtggggcaggacagcaagggggaggattgggaagagaatagcaggcatgctggggaattttgattctcaaacaaatgtgtcacaaagtaaggattctgatgtgtatatcacagacaaaactgtgctagacatgaggtctatggacttcaagagcaacagtgctgtggcctggagcaacaaatctgactttgcatgtgcaaacgccttcaacaacagcattattccagaagacaccttcttccccagcccaggtaagggcagctttggtgccttcgcaggctgtttccttgcttcaggaatggccaggttctgcccagagctctggtcaatgatgtctaaaactcctctgattggtggtctcggccttatccattgccaccaaaaccctctttttactaagaaacagtgagccttgttctggcagtccagagaatgacacgggaaaaaagcagatg

SEQ ID NO: 49 - protein, 580 aa, synthetic construct
MEFGLSWLFLVAILKGVQCRMAQVQLQQSGAELARPGASVKMSCKASGYTFTTYTIHWVRRRPGHDLEWIGYINPSSGCSDYNQNFKGKTTLTADKSSNTAYMQLNSLTSEDSAVYYCARRADYGNYEYTWFAYWGQGTTVTVSSSSGGGGSGGGGSGGGGSVIELTQSPKFMSTSVGDRVNVTYKASQNVGTNVAWFQQKPGQSPKVLIYSASYRYSGVPDRFTGSGSGTDFTLTISNVQSEDLAEYFCQQYHTYPLTFGGGTKLEIKRSDPGDPAESKYGPPCPPCPGQPREPQVYTLPPSRDELTKNQVSLTCLVKGFYPSDIAVEWESNGQPENNYKTTPPVLDSDGSFFLYSKLTVDKSRWQQGNVFSCSVMHEALHNHYTQKSLSLSPGKKDPKFWVLVVVGGVLACYSLLVTVAFIIFWVRSKRSRLLHSDYMNMTPRRPGPTRKHYQPYAPPRDFAAYRSRVKFSRSADAPAYQQGQNQLYNELNLGRREEYDVLDKRRGRDPEMGGKPRRKNPQEGLYNELQKDKMAEAYSEIGMKGERRRGKGHDGLYQGLSTATKDTYDALHMQALPPR

SEQ ID NO: 50 - DNA, 2838 bp, synthetic construct
  source 1..2838: mol_type = other DNA
tattaaataaaagaataagcagtattattaagtagccctgcatttcaggtttccttgagtggcaggccaggcctggccgtgaacgttcactgaaatcatggcctcttggccaagattgatagcttgtgcctgtccctgagtcccagtccatcacgagcagctggtttctaagatgctatttcccgtataaagcatgagaccgtgacttgccagccccacagagccccgcccttgtccatcactggcatctggactccagcctgggttggggcaaagagggaaatgagatcatgtcctaaccctgatcctcttgtcccacagatatccagaaccctgaccctgccgtgtaccagctgagagactctaaatccagtgacaagtctgtctgcctattcaccggcagcggcgccaccaacttcagcctgctgaagcaggccggcgacgtggaagagaaccccgggcccatggagtttggcctgagctggctgtttctggtggccattctgaagggcgtgcagtgccgtatggcccaggttcagctgcagcaatcaggggccgaactcgcccgacctggcgcctccgttaagatgagttgcaaagcctcaggatatacgttcacgacctatactattcactgggttcgccgacggcccggacacgacctggaatggattggctacattaacccctcttcagggtgctcagactataaccaaaatttcaaaggtaaaaccaccctcacggcagataagagtagcaatacagcttatatgcaattgaattccctgactagcgaagattctgcagtctactactgcgccaggcgtgcagattacggaaactacgaatacacatggttcgcttactggggccaagggactactgtgaccgtctcttccagtagcggaggcggaggaagtggtggcggaggttctggcggcggaggatctgtgatcgagttgactcagagccccaaattcatgagtaccagcgttggtgatcgtgttaacgtaacctacaaagcgtctcaaaatgtgggaacaaacgttgcatggtttcagcagaagcccggccagtccccaaaggtcctgatctatagcgctagctaccgttactccggtgttcccgaccggtttaccggaagcggcagtggcacagatttcactctgactatctccaatgtgcagagtgaggatctcgcggaatatttttgtcaacagtatcacacgtaccccctgacttttggggggggcacaaaacttgagataaagcgctcagacccaggggatcccgccgagtctaaatatggcccaccttgcccaccgtgcccagggcagccccgagaaccacaggtgtacaccctgcccccatcccgggatgagctgaccaagaaccaggtcagcctgacctgcctggtcaaaggcttctatcccagcgacatcgccgtggagtgggagagcaatgggcaaccggagaacaactacaagaccacgcctcccgtgctggactccgacggctccttcttcctctacagcaagctcaccgtggacaagagcaggtggcagcaggggaacgtcttctcatgctccgtgatgcatgaggctctgcacaaccactacacgcagaagagcctctccctgtctccgggtaaaaaagatcccaaattttgggtgctggtggtggttggtggagtcctggcttgctatagcttgctagtaacagtggcctttattattttctgggtgaggagtaagaggagcaggctcctgcacagtgactacatgaacatgactccccgccgccccgggcccacccgcaagcattaccagccctatgccccaccacgcgacttcgcagcctatcgctccagagtgaagttcagcaggagcgcagacgcccccgcgtaccagcagggccagaaccagctctataacgagctcaatctaggacgaagagaggagtacgatgttttggacaagagacgtggccgggaccctgagatggggggaaagccgagaaggaagaaccctcaggaaggcctgtacaatgaactgcagaaagataagatggcggaggcctacagtgagattgggatgaaaggcgagcgccggaggggcaaggggcacgatggcctttaccagggtctcagtacagccaccaaggacacctacgacgcccttcacatgcaggccctgccccctcgctgactagagctcgctgatcagcctcgactgtgccttctagttgccagccatctgttgtttgcccctcccccgtgccttccttgaccctggaaggtgccactcccactgtcctttcctaataaaatgaggaaattgcatcgcattgtctgagtaggtgtcattctattctggggggtggggtggggcaggacagcaagggggaggattgggaagagaatagcaggcatgctggggaattttgattctcaaacaaatgtgtcacaaagtaaggattctgatgtgtatatcacagacaaaactgtgctagacatgaggtctatggacttcaagagcaacagtgctgtggcctggagcaacaaatctgactttgcatgtgcaaacgccttcaacaacagcattattccagaagacaccttcttccccagcccaggtaagggcagctttggtgccttcgcaggctgtttccttgcttcaggaatggccaggttctgcccagagctctggtcaatgatgtctaaaactcctctgattggtggtctcggccttatccattgccaccaaaaccctctttttactaagaaacagtgagccttgttctggcagtccagagaatgacacgggaaaaaagcagatg

SEQ ID NO: 51 - protein, 565 aa, synthetic construct
MEFGLSWLFLVAILKGVQCEIVLTQSPATLSLSPGERATLSCRASQSVSSNLAWYQQKPGQAPRLLIYDASNRATGIPARLSGSGSGTDFTLTISSLEPEDFAVYYCQQRSNWPWTFGQGTKVEIKSGGGGSGGGGSGGGGSQVQLQQWGAGLLKPSETLSLTCAVYGGSFSGYYWSWIRQPPGKGLEWIGEINHSGSTKYTPSLKSRVTISVDTSKHQFSLKLSSVTAADTAVYYCARETVYYFDLWGRGTLVTVSSGDPAESKYGPPCPPCPGQPREPQVYTLPPSRDELTKNQVSLTCLVKGFYPSDIAVEWESNGQPENNYKTTPPVLDSDGSFFLYSKLTVDKSRWQQGNVFSCSVMHEALHNHYTQKSLSLSPGKKDPKFWVLVVVGGVLACYSLLVTVAFIIFWVRSKRSRLLHSDYMNMTPRRPGPTRKHYQPYAPPRDFAAYRSRVKFSRSADAPAYQQGQNQLYNELNLGRREEYDVLDKRRGRDPEMGGKPRRKNPQEGLYNELQKDKMAEAYSEIGMKGERRRGKGHDGLYQGLSTATKDTYDALHMQALPPR

SEQ ID NO: 52 - DNA, 2793 bp, synthetic construct
  source 1..2793: mol_type = other DNA
tattaaataaaagaataagcagtattattaagtagccctgcatttcaggtttccttgagtggcaggccaggcctggccgtgaacgttcactgaaatcatggcctcttggccaagattgatagcttgtgcctgtccctgagtcccagtccatcacgagcagctggtttctaagatgctatttcccgtataaagcatgagaccgtgacttgccagccccacagagccccgcccttgtccatcactggcatctggactccagcctgggttggggcaaagagggaaatgagatcatgtcctaaccctgatcctcttgtcccacagatatccagaaccctgaccctgccgtgtaccagctgagagactctaaatccagtgacaagtctgtctgcctattcaccggcagcggcgccaccaacttcagcctgctgaagcaggccggcgacgtggaagagaaccccgggcccatggagtttggcctgagctggctgtttctggtggccattctgaagggcgtgcagtgcgagattgtgctgacacagtctcctgctacattaagtctgtctccgggtgaacgcgccaccctgtcctgtcgtgcatcccaatcagtgagtagcaacctggcatggtaccagcagaaacccgggcaagcgccaagattgctcatctacgatgctagcaaccgggccacaggaataccagcccgacttagcggctctggcagcgggaccgacttcactctcactatctcatccctagagcccgaggacttcgccgtctattattgccagcagaggtcgaattggccttggacctttggccagggaacgaaggttgaaattaagagcggaggcggaggaagtggtggcggaggttctggcggcggaggatctcaggttcagttgcagcaatggggtgccgggctgttgaagccaagtgagaccctctcgttaacctgcgctgtctacggggggagcttttccggatattactggagctggatacgccagccgcctggaaaaggcctggagtggatcggcgaaatcaaccactccggctcaacaaaatacaccccctccctaaagagcagggtgacaatttcagtagacacttctaagcatcaattctcccttaaactgtctagcgtgactgcggctgacactgcagtttactattgtgccagagaaacggtgtattatttcgatctgtggggacggggtaccctcgtgacagtctctagtggggatcccgccgagtctaaatatggcccaccttgcccaccgtgcccagggcagccccgagaaccacaggtgtacaccctgcccccatcccgggatgagctgaccaagaaccaggtcagcctgacctgcctggtcaaaggcttctatcccagcgacatcgccgtggagtgggagagcaatgggcaaccggagaacaactacaagaccacgcctcccgtgctggactccgacggctccttcttcctctacagcaagctcaccgtggacaagagcaggtggcagcaggggaacgtcttctcatgctccgtgatgcatgaggctctgcacaaccactacacgcagaagagcctctccctgtctccgggtaaaaaagatcccaaattttgggtgctggtggtggttggtggagtcctggcttgctatagcttgctagtaacagtggcctttattattttctgggtgaggagtaagaggagcaggctcctgcacagtgactacatgaacatgactccccgccgccccgggcccacccgcaagcattaccagccctatgccccaccacgcgacttcgcagcctatcgctccagagtgaagttcagcaggagcgcagacgcccccgcgtaccagcagggccagaaccagctctataacgagctcaatctaggacgaagagaggagtacgatgttttggacaagagacgtggccgggaccctgagatggggggaaagccgagaaggaagaaccctcaggaaggcctgtacaatgaactgcagaaagataagatggcggaggcctacagtgagattgggatgaaaggcgagcgccggaggggcaaggggcacgatggcctttaccagggtctcagtacagccaccaaggacacctacgacgcccttcacatgcaggccctgccccctcgctgactagagctcgctgatcagcctcgactgtgccttctagttgccagccatctgttgtttgcccctcccccgtgccttccttgaccctggaaggtgccactcccactgtcctttcctaataaaatgaggaaattgcatcgcattgtctgagtaggtgtcattctattctggggggtggggtggggcaggacagcaagggggaggattgggaagagaatagcaggcatgctggggaattttgattctcaaacaaatgtgtcacaaagtaaggattctgatgtgtatatcacagacaaaactgtgctagacatgaggtctatggacttcaagagcaacagtgctgtggcctggagcaacaaatctgactttgcatgtgcaaacgccttcaacaacagcattattccagaagacaccttcttccccagcccaggtaagggcagctttggtgccttcgcaggctgtttccttgcttcaggaatggccaggttctgcccagagctctggtcaatgatgtctaaaactcctctgattggtggtctcggccttatccattgccaccaaaaccctctttttactaagaaacagtgagccttgttctggcagtccagagaatgacacgggaaaaaagcagatg

SEQ ID NO: 53 - RNA, 20 nt, synthetic construct
  source 1..20: mol_type = other RNA
gagaatcaaaatcggtgaat